European Patent Application EP 4 328 239 A1, published February 28, 2024. Title: Immunotherapeutics based on MAGEA1-derived epitopes. Applicant: Max-Delbrueck-Centrum fuer Molekulare Medizin in der Helmholtz-Gemeinschaft. The sequence listing filed with the application follows.

SEQUENCE LISTING (201 sequences)

SEQ ID NO: 1 - protein, 10 aa, Homo sapiens
  REGION 1..10: note = MAGEA1 epitope presented on B*44:03
LAETSYVKVL

SEQ ID NO: 2 - protein, 9 aa, Homo sapiens
  REGION 1..9: note = MAGEA1 epitope presented on B*44:03
EEGPSTSCI

SEQ ID NO: 3 - protein, 10 aa, Homo sapiens
  REGION 1..10: note = MAGEA1 epitope presented on B*44:03
KVADLVGFLL

SEQ ID NO: 4 - protein, 9 aa, Homo sapiens
  REGION 1..9: note = MAGEA1 epitope presented on B*07:02
RVRFFFPSL

SEQ ID NO: 5 - protein, 9 aa, Homo sapiens
  REGION 1..9: note = MAGEA1 epitope presented on B*57:03
KVADLVGFL

SEQ ID NO: 6 - protein, 9 aa, Homo sapiens
  REGION 1..9: note = MAGEA1 epitope presented on A*02:01
KVLEYVIKV

SEQ ID NO: 7 - protein, 9 aa, Homo sapiens
  REGION 1..9: note = MAGEA1 epitope presented on A*03:01
SLFRAVITK

SEQ ID NO: 8 - protein, 10 aa, Homo sapiens
  REGION 1..10: note = MAGEA1 epitope presented on A*26:01
EVYDGREHSA

SEQ ID NO: 9 - protein, 9 aa, Homo sapiens
  REGION 1..9: note = MAGEA1 epitope presented on A*29:02
LVGFLLLKY

SEQ ID NO: 10 - protein, 309 aa, Homo sapiens
  REGION 1..309: note = wtMAGEA1
MSLEQRSLHCKPEEALEAQQEALGLVCVQAATSSSSPLVLGTLEEVPTAGSTDPPQSPQGASAFPTTINFTRQRQPSEGSSSREEEGPSTSCILESLFRAVITKKVADLVGFLLLKYRAREPVTKAEMLESVIKNYKHCFPEIFGKASESLQLVFGIDVKEADPTGHSYVLVTCLGLSYDGLLGDNQIMPKTGFLIIVLVMIAMEGGHAPEEEIWEELSVMEVYDGREHSAYGEPRKLLTQDLVQEKYLEYRQVPDSDPARYEFLWGPRALAETSYVKVLEYVIKVSARVRFFFPSLREAALREEEEGV

SEQ ID NO: 11 - protein, 5 aa, Homo sapiens
  REGION 1..5: note = TCR7 TRA CDR1
SIFNT

SEQ ID NO: 12 - protein, 7 aa, Homo sapiens
  REGION 1..7: note = TCR7 TRA CDR2
LYKAGEL

SEQ ID NO: 13 - protein, 11 aa, Homo sapiens
  REGION 1..11: note = TCR7 TRA CDR3
CAALYGNKLVF

SEQ ID NO: 14 - protein, 128 aa, Homo sapiens
  REGION 1..128: note = TCR 7: variable region of TRA (TRAV-CDR3-TRAJ)(aa)
MLLEHLLIILWMQLTWVSGQQLNQSPQSMFIQEGEDVSMNCTSSSIFNTWLWYKQEPGEGPVLLIALYKAGELTSNGRLTAQFGITRKDSFLNISASIPSDVGIYFCAALYGNKLVFGAGTILRVKSY

SEQ ID NO: 15 - DNA, 384 bp, Homo sapiens
  misc_feature 1..384: note = TCR 7: variable region of TRA (na)
  source 1..384: mol_type = other DNA
atgctgctggaacacctcctgattatcctgtggatgcagctgacctgggtgtccggccagcagctgaatcagtctccccagagcatgttcatccaagaaggcgaggacgtttccatgaattgcaccagcagcagcatcttcaacacctggctgtggtacaagcaagagcccggcgaaggaccagtgctgctgattgccttgtataaggccggcgagctgaccagcaacggcagactgacagcccagttcggcattacccggaaggacagcttcctgaacatcagcgccagcattcccagcgacgtgggcatctacttttgcgccgctctgtacggcaacaagctggtgtttggcgccggaaccatcctgagagtgaagtcctac

SEQ ID NO: 16 - protein, 5 aa, Homo sapiens
  REGION 1..5: note = TCR7 TRB CDR1
SGHRS

SEQ ID NO: 17 - protein, 6 aa, Homo sapiens
  REGION 1..6: note = TCR7 TRB CDR2
YFSETQ

SEQ ID NO: 18 - protein, 13 aa, Homo sapiens
  REGION 1..13: note = TCR7 TRB CDR3
CASSSMGANVLTF

SEQ ID NO: 19 - protein, 131 aa, Homo sapiens
  REGION 1..131: note = TCR 7: variable region of TRB (TRBV-CDR3-TRBJ)(aa)
MGSRLLCWVLLCLLGAGPVKAGVTQTPRYLIKTRGQQVTLSCSPISGHRSVSWYQQTPGQGLQFLFEYFSETQRNKGNFPGRFSGRQFSNSRSEMNVSTLELGDSALYLCASSSMGANVLTFGAGSRLTVL

SEQ ID NO: 20 - DNA, 393 bp, Homo sapiens
  misc_feature 1..393: note = TCR 7: variable region of TRB (na)
  source 1..393: mol_type = other DNA
atgggaagtagactgctttgttgggtgctgctgtgcctgcttggagccggacctgtgaaagctggcgtgacccagacacctagatacctgattaagaccagaggccagcaagtgaccctgagctgctctcctatcagcggccacagaagcgtgtcctggtatcagcagacacctggacagggcctgcagttcctgttcgagtacttcagcgagacacagcggaacaagggcaacttccccggcagattttccggcagacagttcagcaacagccgcagcgagatgaacgtgtccacactggaactgggcgacagcgccctgtatctgtgtgcctcttctagcatgggcgccaacgtgctgacatttggcgctggcagtagactgaccgtgctg

SEQ ID NO: 21 - protein, 6 aa, Homo sapiens
  REGION 1..6: note = TCR8 TRA CDR1
TSGFNG

SEQ ID NO: 22 - protein, 6 aa, Homo sapiens
  REGION 1..6: note = TCR8 TRA CDR2
NVLDGL

SEQ ID NO: 23 - protein, 12 aa, Homo sapiens
  REGION 1..12: note = TCR8 TRA CDR3
CAPSSNTGKLIF

SEQ ID NO: 24 - protein, 127 aa, Homo sapiens
  REGION 1..127: note = TCR 8: variable region of TRA (TRAV-CDR3-TRAJ)(aa)
MWGVFLLYVSMKMGGTTGQNIDQPTEMTATEGAIVQINCTYQTSGFNGLFWYQQHAGEAPTFLSYNVLDGLEEKGRFSSFLSRSKGYSYLLLKELQMKDSASYLCAPSSNTGKLIFGQGTTLQVKPD

SEQ ID NO: 25 - DNA, 381 bp, Homo sapiens
  misc_feature 1..381: note = TCR 8: variable region of TRA (na)
  source 1..381: mol_type = other DNA
atgtggggagtgttcctgctgtacgtgtccatgaagatgggcggcaccaccggccagaacatcgatcagcctacagagatgaccgccaccgagggcgccatcgtgcagatcaattgcacctaccagaccagcggcttcaacggcctgttttggtatcagcagcacgccggcgaggcccctacattcctgagctacaatgtgctggacggcctggaagaaaagggcagattcagcagcttcctgagcagaagcaagggctactcctacctgctgctgaaagaactgcagatgaaggacagcgcctcttacctgtgtgcccctagcagcaataccggcaagctgatctttggccagggcaccactctgcaagtgaagcccgac

SEQ ID NO: 26 - protein, 5 aa, Homo sapiens
  REGION 1..5: note = TCR8 TRB CDR1
SGHNS

SEQ ID NO: 27 - protein, 6 aa, Homo sapiens
  REGION 1..6: note = TCR8 TRB CDR2
FNNNVP

SEQ ID NO: 28 - protein, 12 aa, Homo sapiens
  REGION 1..12: note = TCR8 TRB CDR3
CASSLPQETQYF

SEQ ID NO: 29 - protein, 131 aa, Homo sapiens
  REGION 1..131: note = TCR 8: variable region of TRB (TRBV-CDR3-TRBJ)(aa)
MDSWTFCCVSLCILVAKHTDAGVIQSPRHEVTEMGQEVTLRCKPISGHNSLFWYRQTMMRGLELLIYFNNNVPIDDSGMPEDRFSAKMPNASFSTLKIQPSEPRDSAVYFCASSLPQETQYFGPGTRLLVL

SEQ ID NO: 30 - DNA, 393 bp, Homo sapiens
  misc_feature 1..393: note = TCR 8: variable region of TRB (na)
  source 1..393: mol_type = other DNA
atggatagctggaccttttgttgcgtgtccctgtgcatcctggtggccaagcacacagatgccggcgtgatccagtctcctagacacgaagtgaccgagatgggccaagaagtgaccctgcgctgcaagcctatcagcggccacaatagcctgttctggtacagacagaccatgatgagaggcctggaactgctgatctacttcaacaacaacgtgcccatcgacgacagcggcatgcccgaggatagattcagcgccaagatgcccaacgccagcttcagcaccctgaagatccagcctagcgagcccagagatagcgccgtgtacttttgtgccagcagcctgcctcaagagacacagtactttggccctggcaccagactgctggtgctg

SEQ ID NO: 31 - protein, 6 aa, Homo sapiens
  REGION 1..6: note = TCR6 TRA CDR1
DRGSQS

SEQ ID NO: 32 - protein, 6 aa, Homo sapiens
  REGION 1..6: note = TCR6 TRA CDR2
IYSNGD

SEQ ID NO: 33 - protein, 12 aa, Homo sapiens
  REGION 1..12: note = TCR6 TRA CDR3
CAVSSNTGKLIF

SEQ ID NO: 34 - protein, 132 aa, Homo sapiens
  REGION 1..132: note = TCR 6: variable region of TRA (TRAV-CDR3-TRAJ)(aa)
MKSLRVLLVILWLQLSWVWSQQKEVEQNSGPLSVPEGAIASLNCTYSDRGSQSFFWYRQYSGKSPELIMFIYSNGDKEDGRFTAQLNKASQYVSLLIRDSQPSDSATYLCAVSSNTGKLIFGQGTTLQVKPD

SEQ ID NO: 35 - DNA, 396 bp, Homo sapiens
  misc_feature 1..396: note = TCR 6: variable region of TRA (na)
  source 1..396: mol_type = other DNA
atgaagtccctgagagtgctgctggtcatcctgtggctgcagctgtcttgggtctggtcccagcagaaagaggtggaacagaatagcggccctctgagcgttccagaaggcgctatcgcctctctgaattgcacctacagcgacagaggctcccagagcttcttctggtatcggcagtacagcggcaagagccccgagctgattatgttcatctacagcaacggcgacaaagaggacggccggtttacagcccagctgaacaaagccagccagtatgtgtccctgctgatccgggatagccagccaagcgattctgccacctacctgtgtgccgtgtccagcaataccggcaagctgatctttggccagggcaccacactgcaagtgaagcccgac

SEQ ID NO: 36 - protein, 5 aa, Homo sapiens
  REGION 1..5: note = TCR6 TRB CDR1
SGHNS

SEQ ID NO: 37 - protein, 6 aa, Homo sapiens
  REGION 1..6: note = TCR6 TRB CDR2
FNNNVP

SEQ ID NO: 38 - protein, 15 aa, Homo sapiens
  REGION 1..15: note = TCR6 TRB CDR3
CASKWGQGAGDTQYF

SEQ ID NO: 39 - protein, 134 aa, Homo sapiens
  REGION 1..134: note = TCR 6: variable region of TRB (TRBV-CDR3-TRBJ)(aa)
MDSWTFCCVSLCILVAKHTDAGVIQSPRHEVTEMGQEVTLRCKPISGHNSLFWYRQTMMRGLELLIYFNNNVPIDDSGMPEDRFSAKMPNASFSTLKIQPSEPRDSAVYFCASKWGQGAGDTQYFGPGTRLTVL

SEQ ID NO: 40 - DNA, 402 bp, Homo sapiens
  misc_feature 1..402: note = TCR 6: variable region of TRB (na)
  source 1..402: mol_type = other DNA
atggatagctggaccttttgttgcgtgtccctgtgcatcctggtggccaagcacacagatgccggcgtgatccagtctcctagacacgaagtgaccgagatgggccaagaagtgaccctgcgctgcaagcctatcagcggccacaatagcctgttctggtacagacagaccatgatgagaggcctggaactgctgatctacttcaacaacaacgtgcccatcgacgacagcggcatgcccgaggatagattcagcgccaagatgcccaacgccagcttcagcaccctgaagatccagcctagcgagcccagagatagcgccgtgtacttctgcgcctctaagtggggacaaggcgctggcgatacccagtattttggccctggcaccagactgaccgtgctg

SEQ ID NO: 41 - protein, 5 aa, Homo sapiens
  REGION 1..5: note = TCR5 TRA CDR1
SIFNT

SEQ ID NO: 42 - protein, 7 aa, Homo sapiens
  REGION 1..7: note = TCR5 TRA CDR2
LYKAGEL

SEQ ID NO: 43 - protein, 14 aa, Homo sapiens
  REGION 1..14: note = TCR5 TRA CDR3
CAGLRDNYGQNFVF

SEQ ID NO: 44 - protein, 131 aa, Homo sapiens
  REGION 1..131: note = TCR 5: variable region of TRA (TRAV-CDR3-TRAJ)(aa)
MLLEHLLIILWMQLTWVSGQQLNQSPQSMFIQEGEDVSMNCTSSSIFNTWLWYKQEPGEGPVLLIALYKAGELTSNGRLTAQFGITRKDSFLNISASIPSDVGIYFCAGLRDNYGQNFVFGPGTRLSVLPY

SEQ ID NO: 45 - DNA, 393 bp, Homo sapiens
  misc_feature 1..393: note = TCR 5: variable region of TRA (na)
  source 1..393: mol_type = other DNA
atgctgctggaacatctgctgattatcctgtggatgcagctgacctgggtgtccggccagcagctgaatcagtctccccagagcatgttcatccaagaaggcgaggacgtttccatgaactgcaccagcagcagcatcttcaacacctggctgtggtacaagcaagagcccggcgaaggaccagtgctgctgatcgctctttacaaggccggcgagctgaccagcaacggcagactgactgcccagtttggcattacccggaaggacagcttcctgaacatcagcgccagcattcccagcgacgtgggcatctatttttgtgccggcctgcgggacaactacggccagaattttgtgttcggccctggcaccaggctgagcgtgctgccctat

SEQ ID NO: 46 - protein, 5 aa, Homo sapiens
  REGION 1..5: note = TCR5 TRB CDR1
LNHDA

SEQ ID NO: 47 - protein, 6 aa, Homo sapiens
  REGION 1..6: note = TCR5 TRB CDR2
SQIVND

SEQ ID NO: 48 - protein, 13 aa, Homo sapiens
  REGION 1..13: note = TCR5 TRB CDR3
CASRVGGFEGYTF

SEQ ID NO: 49 - protein, 131 aa, Homo sapiens
  REGION 1..131: note = TCR 5: variable region of TRB (TRBV-CDR3-TRBJ)(aa)
MSNQVLCCVVLCFLGANTVDGGITQSPKYLFRKEGQNVTLSCEQNLNHDAMYWYRQDPGQGLRLIYYSQIVNDFQKGDIAEGYSVSREKKESFPLTVTSAQKNPTAFYLCASRVGGFEGYTFGSGTRLTVV

SEQ ID NO: 50 - DNA, 393 bp, Homo sapiens
  misc_feature 1..393: note = TCR 5: variable region of TRB (aa)
  source 1..393: mol_type = other DNA
atgtctaatcaggtgctgtgttgtgtggtgctgtgcttcctgggcgccaatactgtggatggcggcatcacacagagccccaagtacctgttccggaaagagggccagaacgtcaccctgagctgcgagcagaacctgaaccacgacgccatgtactggtacagacaggaccctggacagggcctgagactgatctactacagccagatcgtgaacgacttccagaagggcgacattgccgagggctacagcgtgtccagagagaagaaagagtcctttccactgaccgtgacaagcgcccagaagaaccctaccgccttctacctgtgtgccagcagagttggcggcttcgagggctatacctttggcagcggcaccagactgacagtggtg

SEQ ID NO: 51 - protein, 5 aa, Homo sapiens
  REGION 1..5: note = TCR18.1 TRA CDR1
TTLSN

SEQ ID NO: 52 - protein, 7 aa, Homo sapiens
  REGION 1..7: note = TCR18.1 TRA CDR2
LVKSGEV

SEQ ID NO: 53 - protein, 13 aa, Homo sapiens
  REGION 1..13: note = TCR18.1 TRA CDR3
CANRDNYGQNFVF

SEQ ID NO: 54 - protein, 130 aa, Homo sapiens
  REGION 1..130: note = TCR 18.1: variable region of TRA (TRAV-CDR3-TRAJ)(aa)
MLLITSMLVLWMQLSQVNGQQVMQIPQYQHVQEGEDFTTYCNSSTTLSNIQWYKQRPGGHPVFLIQLVKSGEVKKQKRLTFQFGEAKKNSSLHITATQTTDVGTYFCANRDNYGQNFVFGPGTRLSVLPY

SEQ ID NO: 55 - DNA, 390 bp, Homo sapiens
  misc_feature 1..390: note = TCR 18.1: variable region of TRA (na)
  source 1..390: mol_type = other DNA
atgctgctgattacctccatgctggtcctgtggatgcagctgagccaagtgaacggccagcaagtgatgcagatccctcagtaccagcatgtgcaagaaggcgaggacttcaccacctactgcaacagcagcacaaccctgagcaacatccagtggtacaagcagaggcctggcgggcaccctgtgtttctgatccagctggtcaagagcggcgaagtgaagaagcagaagcggctgaccttccagttcggcgaggccaagaagaactccagcctgcacatcaccgccacacagaccaccgatgtgggcacctacttttgcgccaaccgggacaactacggccagaacttcgtgttcggaccaggcacaagactgtccgtgctgccctac

SEQ ID NO: 56 - protein, 5 aa, Homo sapiens
  REGION 1..5: note = TCR18.1 TRB CDR1
MNHEY

SEQ ID NO: 57 - protein, 6 aa, Homo sapiens
  REGION 1..6: note = TCR18.1 TRB CDR2
SMNVEV

SEQ ID NO: 58 - protein, 15 aa, Homo sapiens
  REGION 1..15: note = TCR18.1 TRB CDR3
CASSRTSGISYEQYF

SEQ ID NO: 59 - protein, 132 aa, Homo sapiens
  REGION 1..132: note = TCR 18.1: variable region of TRB (TRBV-CDR3-TRBJ)(aa)
MGPQLLGYVVLCLLGAGPLEAQVTQNPRYLITVTGKKLTVTCSQNMNHEYMSWYRQDPGLGLRQIYYSMNVEVTDKGDVPEGYKVSRKEKRNFPLILESPSPNQTSLYFCASSRTSGISYEQYGPGTRLTVT

SEQ ID NO: 60 - DNA, 399 bp, Homo sapiens
  misc_feature 1..399: note = TCR 18.1: variable region of TRB (na)
  source 1..399: mol_type = other DNA
atgggacctcaactgctgggatatgtggtgctgtgtctgctcggagccggacctctggaagctcaagtgacacagaaccccagatacctgattaccgtgaccggcaagaaactgaccgtgacctgcagccagaacatgaaccacgagtacatgagctggtacagacaggaccctggcctgggcctgagacagatctactacagcatgaacgtggaagtgaccgacaagggcgacgtgcccgagggctataaggtgtcccggaaagagaagcggaacttcccactgatcctggaaagcccatctcctaaccagaccagcctgtacttctgcgccagcagcagaacaagcggcatcagctacgagcagtacttcggccctggcaccagactgacagtgacc

SEQ ID NO: 61 - protein, 5 aa, Homo sapiens
  REGION 1..5: note = TCR 18.2 TRA CDR1
TTLSN

SEQ ID NO: 62 - protein, 7 aa, Homo sapiens
  REGION 1..7: note = TCR 18.2 TRA CDR2
LVKSGEV

SEQ ID NO: 63 - protein, 13 aa, Homo sapiens
  REGION 1..13: note = TCR 18.2 TRA CDR3
CANRDNYGQNFVF

SEQ ID NO: 64 - protein, 130 aa, Homo sapiens; identical to SEQ ID NO: 54

SEQ ID NO: 65 - DNA, 390 bp, Homo sapiens
  misc_feature 1..390: note = TCR 18.2: variable region of TRA (aa)
  source 1..390: mol_type = other DNA
atgctgctgattacctccatgctggtcctgtggatgcagctgagccaagtgaacggccagcaagtgatgcagatccctcagtaccagcatgtgcaagaaggcgaggacttcaccacctactgcaacagcagcacaaccctgagcaacatccagtggtacaagcagaggccaggcggacaccccgtgtttctgatccagctggtcaagagcggcgaagtgaagaagcagaagcggctgaccttccagttcggcgaggccaagaagaactccagcctgcacatcaccgccacacagaccaccgatgtgggcacctacttttgcgccaaccgggacaactacggccagaacttcgtgttcggccctggcacaagactgagcgtgctgccctac

SEQ ID NO: 66 - protein, 5 aa, Homo sapiens
  REGION 1..5: note = TCR 18.2 TRB CDR1
MNHEY

SEQ ID NO: 67 - protein, 6 aa, Homo sapiens
  REGION 1..6: note = TCR 18.2 TRB CDR2
SMNVEV

SEQ ID NO: 68 - protein, 14 aa, Homo sapiens
  REGION 1..14: note = TCR 18.2 TRB CDR3
CASTRTGTLPEAFF

SEQ ID NO: 69 - protein, 132 aa, Homo sapiens
  REGION 1..132: note = TCR 18.2: variable region of TRB (TRBV-CDR3-TRBJ)(aa)
MGPQLLGYVVLCLLGAGPLEAQVTQNPRYLITVTGKKLTVTCSQNMNHEYMSWYRQDPGLGLRQIYYSMNVEVTDKGDVPEGYKVSRKEKRNFPLILESPSPNQTSLYFCASTRTGTLPEAFFGQGTRLTVV

SEQ ID NO: 70 - DNA, 396 bp, Homo sapiens
  misc_feature 1..396: note = TCR 18.2: variable region of TRB (na)
  source 1..396: mol_type = other DNA
atgggacctcaactgctgggatatgtggtgctgtgtctgctcggagccggacctctggaagctcaagtgacacagaaccccagatacctgattaccgtgaccggcaagaaactgaccgtgacctgcagccagaacatgaaccacgagtacatgagctggtacagacaggaccctggcctgggcctgagacagatctactacagcatgaacgtggaagtgaccgacaagggcgacgtgcccgagggctataaggtgtcccggaaagagaagcggaacttcccactgatcctggaaagcccatctcctaaccagaccagcctgtacttctgcgccagcaccagaaccggaacactgcccgaggccttttttggccaaggcaccagactgacagtggtg

SEQ ID NO: 71 - protein, 7 aa, Homo sapiens
  REGION 1..7: note = TCR23 TRA CDR1
TRDTTYY

SEQ ID NO: 72 - protein, 8 aa, Homo sapiens
  REGION 1..8: note = TCR23 TRA CDR2
RNSFDEQN

SEQ ID NO: 73 - protein, 14 aa, Homo sapiens
  REGION 1..14: note = TCR23 TRA CDR3
CALSVTYTGNQFYF

SEQ ID NO: 74 - protein, 136 aa, Homo sapiens
  REGION 1..136: note = TCR 23: variable region of TRA (TRAV-CDR3-TRAJ)(aa)
MLTASLLRAVIASICVVSSMAQKVTQAQTEISVVEKEDVTLDCVYETRDTTYYLFWYKQPPSGELVFLIRRNSFDEQNEISGRYSWNFQKSTSSFNFTITASQVVDSAVYFCALSVTYTGNQFYFGTGTSLTVIPN

SEQ ID NO: 75 - DNA, 408 bp, Homo sapiens
  misc_feature 1..408: note = TCR 23: variable region of TRA (na)
  source 1..408: mol_type = other DNA
atgctgacagcctctctgctgagagccgtgatcgccagcatctgtgtggtgtctagcatggcccagaaagtgacacaggcccagaccgagatcagcgtggtggaaaaagaagatgtgaccctggactgcgtgtacgagacacgggacaccacctactacctgttctggtacaagcagcctcctagcggcgagctggtgttcctgattcggagaaacagcttcgacgagcagaacgagatctccggccggtacagctggaacttccagaagtccaccagcagcttcaacttcaccatcaccgccagccaggtggtggattccgccgtgtatttttgcgccctgtccgtgacctacaccggcaaccagttctactttggcaccggcacaagcctgacagtgatccccaac

SEQ ID NO: 76 - protein, 5 aa, Homo sapiens
  REGION 1..5: note = TCR23 TRB CDR1
SGDLS

SEQ ID NO: 77 - protein, 6 aa, Homo sapiens
  REGION 1..6: note = TCR23 TRB CDR2
YYNGEE

SEQ ID NO: 78 - protein, 15 aa, Homo sapiens
  REGION 1..15: note = TCR23 TRB CDR3
CASSVQGQGTDTQYF

SEQ ID NO: 79 - protein, 133 aa, Homo sapiens
  REGION 1..133: note = TCR 23: variable region of TRB (TRBV-CDR3-TRBJ)(aa)
MGFRLLCCVAFCLLGAGPVDSGVTQTPKHLITATGQRVTLRCSPRSGDLSVYWYQQSLDQGLQFLIQYYNGEERAKGNILERFSAQQFPDLHSELNLSSLELGDSALYFCASSVQGQGTDTQYFGPGTRLTVL

SEQ ID NO: 80 - DNA, 399 bp, Homo sapiens
  misc_feature 1..399: note = TCR 23: variable region of TRB (na)
  source 1..399: mol_type = other DNA
atgggttttagactgctgtgctgcgtggccttctgtctgcttggagctggccctgtggatagcggcgttacccagacacctaagcacctgattacagccaccggccagcgcgtgaccctgagatgttctcctagaagcggcgacctgagcgtgtactggtatcagcagtctctggaccagggcctgcagttcctgatccagtactacaacggcgaggaaagagccaagggcaacatcctggaacggttcagcgcccagcagttcccagatctgcacagcgagctgaacctgagcagcctggaactgggagatagcgccctgtacttctgtgccagctctgtgcaaggccagggcaccgacacacagtattttggccctggcaccagactgaccgtgctg

SEQ ID NO: 81 - protein, 7 aa, Homo sapiens
  REGION 1..7: note = TCR19 TRA CDR1
TSENNYY

SEQ ID NO: 82 - protein, 8 aa, Homo sapiens
  REGION 1..8: note = TCR19 TRA CDR2
QEAYKQQN

SEQ ID NO: 83 - protein, 12 aa, Homo sapiens
  REGION 1..12: note = TCR19 TRA CDR3
CAFISGYSTLTF

SEQ ID NO: 84 - protein, 134 aa, Homo sapiens
  REGION 1..134: note = TCR 19: variable region of TRA (TRAV-CDR3-TRAJ)(aa)
MTRVSLLWAVVVSTCLESGMAQTVTQSQPEMSVQEAETVTLSCTYDTSENNYYLFWYKQPPSRQMILVIRQEAYKQQNATENRFSVNFQKAAKSFSLKISDSQLGDTAMYFCAFISGYSTLTFGKGTMLLVSPD

SEQ ID NO: 85 - DNA, 402 bp, Homo sapiens
  misc_feature 1..402: note = TCR 19: variable region of TRA (na)
  source 1..402: mol_type = other DNA
atgaccagagtgtctctgctgtgggccgtcgtggtgtccacctgtctggaatctggaatggcccagaccgtgacacagtcccagcctgagatgtctgtgcaagaggccgagactgtgaccctgagctgcacctacgataccagcgagaacaactactacctgttctggtacaagcagcctcctagccggcagatgatcctggtcatcagacaagaggcctataagcagcagaacgccaccgagaacagattcagcgtgaacttccagaaggccgccaagagctttagcctgaagatcagcgatagccagctgggcgacaccgccatgtacttttgtgccttcatcagcggctacagcaccctgacctttggcaagggcacaatgctgctcgtgtccccagac

SEQ ID NO: 86 - protein, 5 aa, Homo sapiens
  REGION 1..5: note = TCR19 TRB CDR1
MNHEY

SEQ ID NO: 87 - protein, 6 aa, Homo sapiens
  REGION 1..6: note = TCR19 TRB CDR2
SMNVEV

SEQ ID NO: 88 - protein, 15 aa, Homo sapiens
  REGION 1..15: note = TCR19 TRB CDR3
CASRTSHPQTYEQYF

SEQ ID NO: 89 - protein, 133 aa, Homo sapiens
  REGION 1..133: note = TCR 19: variable region of TRB (TRBV-CDR3-TRBJ)(aa)
MGPQLLGYVVLCLLGAGPLEAQVTQNPRYLITVTGKKLTVTCSQNMNHEYMSWYRQDPGLGLRQIYYSMNVEVTDKGDVPEGYKVSRKEKRNFPLILESPSPNQTSLYFCASRTSHPQTYEQYFGPGTRLTVT

SEQ ID NO: 90 - DNA, 399 bp, Homo sapiens
  misc_feature 1..399: note = TCR 19: variable region of TRB (na)
  source 1..399: mol_type = other DNA
atgggacctcaactgctgggatatgtggtgctgtgtctgctcggagccggacctctggaagctcaagtgacacagaaccccagatacctgattaccgtgaccggcaagaaactgaccgtgacctgcagccagaacatgaaccacgagtacatgagctggtacagacaggaccctggcctgggcctgagacagatctactacagcatgaacgtggaagtgaccgacaagggcgacgtgcccgagggctataaggtgtcccggaaagagaagcggaacttcccactgatcctggaaagcccatctcctaaccagaccagcctgtacttctgcgccagcagaaccagccatcctcagacctacgagcagtacttcggccctggcaccagactgacagtgacc

SEQ ID NO: 91 - protein, 6 aa, Homo sapiens
  REGION 1..6: note = TCR1 TRA CDR1
ATGYPS

SEQ ID NO: 92 - protein, 7 aa, Homo sapiens
  REGION 1..7: note = TCR1 TRA CDR2
ATKADDK

SEQ ID NO: 93 - protein, 13 aa, Homo sapiens
  REGION 1..13: note = TCR1 TRA CDR3
CALSGGGSYIPTF

SEQ ID NO: 94 - protein, 132 aa, Homo sapiens
  REGION 1..132: note = TCR 1: variable region of TRA (TRAV-CDR3-TRAJ)(aa)
MNYSPGLVSLILLLLGRTRGNSVTQMEGPVTLSEEAFLTINCTYTATGYPSLFWYVQYPGEGLQLLLKATKADDKGSNKGFEATYRKETTSFHLEKGSVQVSDSAVYFCALSGGGSYIPTFGRGTSLIVHPY

SEQ ID NO: 95 - DNA, 396 bp, Homo sapiens
  misc_feature 1..396: note = TCR 1: variable region of TRA (na)
  source 1..396: mol_type = other DNA
atgaattacagccccggactggtgtctctgattctgctgctgctgggaagaaccagaggcaacagcgtgacccagatggaaggcccagtgactctgagcgaggaagccttcctgaccatcaattgcacctacaccgccacaggctaccccagcctgttttggtacgtgcagtatcctggcgagggcctgcagctgctgcttaaggccacaaaggccgacgacaagggcagcaacaagggctttgaggccacctaccggaaagagacaaccagcttccacctggaaaagggcagcgtccaggtgtccgattctgccgtgtatttctgcgccctgtctggcggcggaagctacatccctacatttggcagaggcacaagcctgatcgtgcacccctac

SEQ ID NO: 96 - protein, 5 aa, Homo sapiens
  REGION 1..5: note = TCR1 TRB CDR1
SGHAT

SEQ ID NO: 97 - protein, 6 aa, Homo sapiens
  REGION 1..6: note = TCR1 TRB CDR2
FQNNGV

SEQ ID NO: 98 - protein, 15 aa, Homo sapiens
CASSSPGQLNTEAFF

SEQ ID NO: 99 - protein, 134 aa, Homo sapiens
  REGION 1..134: note = TCR 1: variable region of TRB (TRBV-CDR3-TRBJ)(aa)
MGTRLLCWAALCLLGAELTEAGVAQSPRYKIIEKRQSVAFWCNPISGHATLYWYQQILGQGPKLLIQFQNNGVVDDSQLPKDRFSAERLKGVDSTLKIQPAKLEDSAVYLCASSSPGQLNTEAFFGQGTRLTVV

SEQ ID NO: 100 - DNA, 402 bp, Homo sapiens
  misc_feature 1..402: note = TCR 1: variable region of TRB (na)
  source 1..402: mol_type = other DNA
atgggaacaagattgctttgttgggccgctctgtgtctgctgggagccgaacttacagaagccggcgttgcccagtctcctcggtacaagatcatcgagaagcggcagagcgtggccttctggtgcaatcctatctctggccacgccacactgtactggtatcagcagatcctcggccagggacctaagctgctgattcagttccagaacaacggcgtggtggacgacagccagctgcctaaggatagattcagcgccgagcggctgaaaggcgtggacagcacactgaagatccagcctgccaagctggaagatagcgccgtgtacctgtgtgcctctagctctcctggccagctgaacaccgaggccttttttggccaaggcaccagactgaccgtggtg

SEQ ID NO: 101 - protein, 6 aa, Homo sapiens
  REGION 1..6: note = TCR20 TRA CDR1
DRGSQS

SEQ ID NO: 102 - protein, 6 aa, Homo sapiens
  REGION 1..6: note = TCR20 TRA CDR2
IYSNGD

SEQ ID NO: 103 - protein, 15 aa, Homo sapiens
  REGION 1..15: note = TCR20 TRA CDR3
CAVNAPRPGYSTLTF

SEQ ID NO: 104 - protein, 135 aa, Homo sapiens
  REGION 1..135: note = TCR 20: variable region of TRA (TRAV-CDR3-TRAJ)(aa)
MKSLRVLLVILWLQLSWVWSQQKEVEQNSGPLSVPEGAIASLNCTYSDRGSQSFFWYRQYSGKSPELIMFIYSNGDKEDGRFTAQLNKASQYVSLLIRDSQPSDSATYLCAVNAPRPGYSTLTFGKGTMLLVSPE

SEQ ID NO: 105 - DNA, 405 bp, Homo sapiens
  misc_feature 1..405: note = TCR 20: variable region of TRA (na)
  source 1..405: mol_type = other DNA
atgaagtccctgagagtgctgctggtcatcctgtggctgcagctgtcttgggtctggtcccagcagaaagaggtggaacagaatagcggccctctgagcgttccagaaggcgctatcgccagcctgaattgcacctacagcgacagaggctcccagagcttcttctggtatcggcagtacagcggcaagagccccgagctgattatgttcatctacagcaacggcgacaaagaggacggccggtttacagcccagctgaacaaggccagccagtacgtgtccctgctgatccgggatagccagcctagcgattctgccacatatctgtgcgccgtgaacgcccctagacctggctacagcacactgacctttggcaagggcaccatgctgctcgtgtccccagag

SEQ ID NO: 106 - protein, 5 aa, Homo sapiens
  REGION 1..5: note = TCR20 TRB CDR1
MDHEN

SEQ ID NO: 107 - protein, 6 aa, Homo sapiens
  REGION 1..6: note = TCR20 TRB CDR2
SYDVKM

SEQ ID NO: 108 - protein, 13 aa, Homo sapiens
  REGION 1..13: note = TCR20 TRB CDR3
CASSLSMNTEAFF

SEQ ID NO: 109 - protein, 131 aa, Homo sapiens
  REGION 1..131: note = TCR 20: variable region of TRB (TRBV-CDR3-TRBJ)(aa)
MGIRLLCRVAFCFLAVGLVDVKVTQSSRYLVKRTGEKVFLECVQDMDHENMFWYRQDPGLGLRLIYFSYDVKMKEKGDIPEGYSVSREKKERFSLILESASTNQTSMYLCASSLSMNTEAFFGQGTRLTVV

SEQ ID NO: 110 - DNA, 393 bp, Homo sapiens
  misc_feature 1..393: note = TCR 20: variable region of TRB (na)
  source 1..393: mol_type = other DNA
atgggaattagactgctgtgcagagtggccttctgcttcctggctgttggcctggtggacgtgaaagtgacccagagcagcagatacctggtcaagagaaccggcgagaaggtgttcctggaatgcgtgcaggacatggaccacgagaatatgttctggtacagacaggaccccggcctgggcctgagactgatctacttcagctacgacgtgaagatgaaggaaaagggcgacatccccgagggctacagcgtgtccagagagaagaaagagcggttcagcctgatcctggaaagcgccagcaccaaccagaccagcatgtacctgtgtgccagcagcctgtctatgaacaccgaggcctttttcggccaaggcaccagactgaccgtggtg

SEQ ID NO: 111 - protein, 5 aa, Homo sapiens
  REGION 1..5: note = TCR22 TRA CDR1
TSINN

SEQ ID NO: 112 - protein, 7 aa, Homo sapiens
  REGION 1..7: note = TCR22 TRA CDR2
IRSNERE

SEQ ID NO: 113 - protein, 13 aa, Homo sapiens
  REGION 1..13: note = TCR22 TRA CDR3
CATDEGGAQKLVF

SEQ ID NO: 114 - protein, 132 aa, Homo sapiens
  REGION 1..132: note = TCR 22: variable region of TRA (TRAV-CDR3-TRAJ)(aa)
METLLGVSLVILWLQLARVNSQQGEEDPQALSIQEGENATMNCSYKTSINNLQWYRQNSGRGLVHLILIRSNEREKHSGRLRVTLDTSKKSSSLLITASRAADTASYFCATDEGGAQKLVFGQGTRLTINPN

SEQ ID NO: 115 - DNA, 396 bp, Homo sapiens
  misc_feature 1..396: note = TCR 22: variable region of TRA (na)
  source 1..396: mol_type = other DNA
atggaaacactgctgggcgtgtccctggtcatcctgtggctgcaactggctagagtgaacagccagcagggcgaagaagatcctcaggctctgagcatccaagagggcgagaacgccaccatgaactgcagctacaagacctccatcaacaacctgcagtggtacaggcagaactctggcagaggcctggtgcacctgattctgatccggtccaacgagagagagaagcactccggcagactgcgcgtgaccctggacacaagcaagaagtctagctccctgctgattaccgccagcagagccgccgatacagccagctacttttgcgccactgatgaaggcggagcccagaaactggtgttcggccagggaacaagactgaccatcaatcccaac

SEQ ID NO: 116 - protein, 5 aa, Homo sapiens
  REGION 1..5: note = TCR22 TRB CDR1
MDHEN

SEQ ID NO: 117 - protein, 6 aa, Homo sapiens
  REGION 1..6: note = TCR22 TRB CDR2
SYDVKM

SEQ ID NO: 118 - protein, 15 aa, Homo sapiens
  REGION 1..15: note = TCR22 TRB CDR3
CATVGRGEDRGEQFF

SEQ ID NO: 119 - protein, 133 aa, Homo sapiens
  REGION 1..133: note = TCR 22: variable region of TRB (TRBV-CDR3-TRBJ)(aa)
MGIRLLCRVAFCFLAVGLVDVKVTQSSRYLVKRTGEKVFLECVQDMDHENMFWYRQDPGLGLRLIYFSYDVKMKEKGDIPEGYSVSREKKERFSLILESASTNQTSMYLCATVGRGEDRGEQFFGPGTRLTVL

SEQ ID NO: 120 - DNA, 399 bp, Homo sapiens
  misc_feature 1..399: note = TCR 22: variable region of TRB (na)
  source 1..399: mol_type = other DNA
atgggaattagactgctgtgcagagtggccttctgcttcctggctgttggcctggtggacgtgaaagtgacccagagcagcagatacctggtcaagagaaccggcgagaaggtgttcctggaatgcgtgcaggacatggaccacgagaatatgttctggtacagacaggaccccggcctgggcctgagactgatctacttcagctacgacgtgaagatgaaggaaaagggcgacatccccgagggctacagcgtgtccagagagaagaaagagcggttcagcctgatcctggaaagcgccagcaccaaccagaccagcatgtacctgtgtgccacagtcggcagaggcgaggatagaggcgagcagttttttggccctggcaccagactgaccgtgctg

SEQ ID NO: 121 - protein, 6 aa, Homo sapiens
  REGION 1..6: note = TCR24 TRA CDR1
VSPFSN

SEQ ID NO: 122 - protein, 7 aa, Homo sapiens
  REGION 1..7: note = TCR24 TRA CDR2
MTFSENT

SEQ ID NO: 123 - protein, 13 aa, Homo sapiens
  REGION 1..13: note = TCR24 TRA CDR3
CVVSNNAGNMLTF

SEQ ID NO: 124 - protein, 134 aa, Homo sapiens
  REGION 1..134: note = TCR 24: variable region of TRA (TRAV-CDR3-TRAJ)(aa)
MKKHLTTFLVILWLYFYRGNGKNQVEQSPQSLIILEGKNCTLQCNYTVSPFSNLRWYKQDTGRGPVSLTIMTFSENTKSNGRYTATLDADTKQSSLHITASQLSDSASYICVVSNNAGNMLTFGGGTRLMVKPH

SEQ ID NO: 125 - DNA, 402 bp, Homo sapiens
  misc_feature 1..402: note = TCR 24: variable region of TRA (na)
  source 1..402: mol_type = other DNA
atgaagaagcacctgaccacctttctggtcatcctgtggctgtacttctacagaggcaacggcaagaaccaggtggaacagagcccacagagcctgattatcctggaaggcaagaactgcaccctgcagtgcaactacaccgtgtctcccttcagcaacctgcggtggtacaagcaggatacaggcagaggcccagtgtctctgaccatcatgaccttcagcgagaacaccaagagcaacggccggtacaccgccacactggatgccgatacaaagcagtccagcctgcacatcacagccagccagctgagcgatagcgcctcctacatctgcgtggtgtccaacaacgccggcaacatgctgacatttggcggcggaacccggctgatggtcaagccccat

SEQ ID NO: 126 - protein, 5 aa, Homo sapiens
  REGION 1..5: note = TCR24 TRB CDR1
LNHNV

SEQ ID NO: 127 - protein, 6 aa, Homo sapiens
  REGION 1..6: note = TCR24 TRB CDR2
YYDKDF

SEQ ID NO: 128 - protein, 15 aa, Homo sapiens
  REGION 1..15: note = TCR24 TRB CDR3
CATSRESLGRDEQFF

SEQ ID NO: 129 - protein, 133 aa, Homo sapiens
  REGION 1..133: note = TCR 24: variable region of TRB (TRBV-CDR3-TRBJ)(aa)
MGPGLLHWMALCLLGTGHGDAMVIQNPRYQVTQFGKPVTLSCSQTLNHNVMYWYQQKSSQAPKLLFHYYDKDFNNEADTPDNFQSRRPNTSFCFLDIRSPGLGDTAMYLCATSRESLGRDEQFFGPGTRLTVL

SEQ ID NO: 130 - DNA, 399 bp, Homo sapiens
  misc_feature 1..399: note = TCR 24: variable region of TRB (na)
  source 1..399: mol_type = other DNA
atgggacctggattgcttcattggatggccctgtgtctgctcggcacaggacatggcgacgctatggtcattcagaaccccagataccaagtgacccagttcggcaagcccgtgacactgagctgtagccagacactgaaccacaacgtgatgtactggtatcagcagaagtcctctcaggcccctaagctgctgttccactactacgacaaggacttcaacaacgaggccgacacacccgacaacttccagagcagaaggcccaataccagcttctgcttcctggacatcagaagccctggcctgggcgatacagccatgtatctgtgtgccaccagcagagagtctctcggcagggacgagcagtttttcggccctggcacaagactgaccgtgctg

SEQ ID NO: 131 - protein, 7 aa, Homo sapiens
  REGION 1..7: note = TCR2 TRA CDR1
TSDPSYG

SEQ ID NO: 132 - protein, 8 aa, Homo sapiens
  REGION 1..8: note = TCR2 TRA CDR2
QGSYDQQN

SEQ ID NO: 133 - protein, 13 aa, Homo sapiens
  REGION 1..13: note = TCR2 TRA CDR3
CASREGSARQLTF

SEQ ID NO: 134 - protein, 135 aa, Homo sapiens
  REGION 1..135: note = TCR 2: variable region of TRA (TRAV-CDR3-TRAJ)(aa)
MSLSSLLKVVTASLWLGPGIAQKITQTQPGMFVQEKEAVTLDCTYDTSDPSYGLFWYKQPSSGEMIFLIYQGSYDQQNATEGRYSLNFQKARKSANLVISASQLGDSAMYFCASREGSARQLTFGSGTQLTVLPD

SEQ ID NO: 135 - DNA, 405 bp, Homo sapiens
  misc_feature 1..405: note = TCR 2: variable region of TRA (na)
  source 1..405: mol_type = other DNA
atgtctctgtctagcctgctgaaggtggtcaccgccagtctgtggctcggacctggaatcgcccagaagatcacccagacacagcccggcatgttcgtgcaagagaaagaagctgtgaccctggactgcacctacgacaccagcgatcctagctacggactgttttggtacaagcagcccagcagcggcgagatgatcttcctgatctaccagggctcctacgaccagcagaatgccaccgagggcagatacagcctgaacttccagaaggcccggaagtccgccaacctggtcatttctgctagccagctgggcgactccgccatgtacttttgcgctagcagagagggcagcgccagacagctgacatttggctctggaacccagctcacagtgctgcccgac

SEQ ID NO: 136 - protein, 5 aa, Homo sapiens
  REGION 1..5: note = TCR2 TRB CDR1
MDHEN

SEQ ID NO: 137 - protein, 6 aa, Homo sapiens
  REGION 1..6: note = TCR2 TRB CDR2
SYDVKM

SEQ ID NO: 138 - protein, 11 aa, Homo sapiens
  REGION 1..11: note = TCR2 TRB CDR3
CASDSADTQYF

SEQ ID NO: 139 - protein, 129 aa, Homo sapiens
  REGION 1..129: note = TCR 2: variable region of TRB (TRBV-CDR3-TRBJ)(aa)
MGIRLLCRVAFCFLAVGLVDVKVTQSSRYLVKRTGEKVFLECVQDMDHENMFWYRQDPGLGLRLIYFSYDVKMKEKGDIPEGYSVSREKKERFSLILESASTNQTSMYLCASDSADTQYFGPGTRLTVL

SEQ ID NO: 140 - DNA, 387 bp, Homo sapiens
  misc_feature 1..387: note = TCR 2: variable region of TRB (na)
  source 1..387: mol_type = other DNA
atgggaattagactgctgtgcagagtggccttctgcttcctggctgttggcctggtggacgtgaaagtgacccagagcagcagatacctggtcaagagaaccggcgagaaggtgttcctggaatgcgtgcaggacatggaccacgagaatatgttctggtacagacaggaccccggcctgggcctgagactgatctacttcagctacgacgtgaagatgaaggaaaagggcgacatccccgagggctacagcgtgtccagagagaagaaagagcggttcagcctgatcctggaaagcgccagcaccaaccagaccagcatgtacctgtgtgccagcgacagcgccgacacacagtattttggccctggcaccagactgaccgtgctg

SEQ ID NO: 141 - protein, 6 aa, Homo sapiens
  REGION 1..6: note = TCR4 TRA CDR1
SSVPPY

SEQ ID NO: 142 - protein, 8 aa, Homo sapiens
  REGION 1..8: note = TCR4 TRA CDR2
YTSAATLV

SEQ ID NO: 143 - protein, 13 aa, Homo sapiens
  REGION 1..13: note = TCR4 TRA CDR3
CAVSNSGNTPLVF

SEQ ID NO: 144 - protein, 133 aa, Homo sapiens
  REGION 1..133: note = TCR 4: variable region of TRA (TRAV-CDR3-TRAJ)(aa)
MLLLLVPVLEVIFTLGGTRAQSVTQLGSHVSVSEGALVLLRCNYSSSVPPYLFWYVQYPNQGLQLLLKYTSAATLVKGINGFEAEFKKSETSFHLTKPSAHMSDAAEYFCAVSNSGNTPLVFGKGTRLSVIAN

SEQ ID NO: 145 - DNA, 399 bp, Homo sapiens
  misc_feature 1..399: note = TCR 4: variable region of TRA (na)
  source 1..399: mol_type = other DNA
atgctgcttctgctggtgcctgtgctggaagtgatctttaccctcggcggcactagagcccagagcgttacacagctgggcagccatgtgtccgtgtctgaaggtgctctggtgctgctgagatgcaactactccagcagcgtgccaccttacctgttttggtacgtgcagtaccccaaccagggcctgcaactgctgctgaagtacacatctgccgccacactggtcaagggcatcaatggcttcgaggccgagttcaagaagtccgagacaagcttccacctgaccaagcctagcgctcacatgtccgatgccgccgaatacttctgcgccgtgtccaactctggcaacacccctctggtgtttggcaaaggcacccggctgagcgtgatcgccaat

SEQ ID NO: 146 - protein, 5 aa, Homo sapiens
  REGION 1..5: note = TCR4 TRB CDR1
PRHDT

SEQ ID NO: 147 - protein, 6 aa, Homo sapiens
  REGION 1..6: note = TCR4 TRB CDR2
FYEKMQ

SEQ ID NO: 148 - protein, 13 aa, Homo sapiens
  REGION 1..13: note = TCR4 TRB CDR3
CASSSTTGDGYTF

SEQ ID NO: 149 - protein, 141 aa, Homo sapiens
  REGION 1..141: note = TCR 4: variable region of TRB (TRBV-CDR3-TRBJ)(aa)
MLSPDLPDSAWNTRLLCHVMLCLLGAVSVAAGVIQSPRHLIKEKRETATLKCYPIPRHDTVYWYQQGPGQDPQFLISFYEKMQSDKGSIPDRFSAQQFSDYHSELNMSSLELGDSALYFCASSSTTGDGYTFGSGTRLTVV

SEQ ID NO: 150 - DNA, 423 bp, Homo sapiens
  misc_feature 1..423: note = TCR 4: variable region of TRB (na)
  source 1..423: mol_type = other DNA
atgctttctccagatctgcctgatagcgcctggaacaccagactgctgtgccatgtgatgctgtgtctgctgggagccgtgtctgttgccgctggcgttatccagtctcctcggcacctcatcaaagagaagagagagacagccacactgaagtgctaccccattccacggcacgacaccgtgtactggtatcagcaaggcccaggccaggatcctcagttcctgattagcttctacgagaagatgcagagcgacaagggcagcatccccgacagattttctgcccagcagttcagcgactaccacagcgagctgaacatgagcagcctggaactgggcgatagcgccctgtacttttgtgccagcagcagcacaacaggcgacggctacacatttggcagcggcacaagactgaccgtggtg

SEQ ID NO: 151 - protein, 9 aa, Homo sapiens
  REGION 1..9: note = MAGEA1 peptide
VADLVGFLL

SEQ ID NO: 152 - protein, 10 aa, Homo sapiens
  REGION 1..10: note = MAGEA1 peptide
DLVGFLLLKY

SEQ ID NO: 153 - protein, 9 aa, Homo sapiens
  REGION 1..9: note = MAGEA1 peptide
AETSYVKVL

SEQ ID NO: 154 - protein, 10 aa, Homo sapiens
  REGION 1..10: note = MAGEA1 peptide
AETSYVKVLE

SEQ ID NO: 155 - protein, 10 aa, Homo sapiens
  REGION 1..10: note = MAGEA1 peptide
ALAETSYVKV

SEQ ID NO: 156 - protein, 9 aa, Homo sapiens
  REGION 1..9: note = MAGEA1 peptide
VADLVGFLL

SEQ ID NO: 157 - protein, 10 aa, Homo sapiens
  REGION 1..10: note = MAGEA1 peptide
ADLVGFLLLK

SEQ ID NO: 158 - protein, 10 aa, Homo sapiens
  REGION 1..10: note = MAGEA1 peptide
AETSYVKVLE

SEQ ID NO: 159 - protein, 9 aa, Homo sapiens
  REGION 1..9: note = MAGEA1 peptide
LEYVIKVSA

SEQ ID NO: 160 - protein, 10 aa, Homo sapiens
  REGION 1..10: note = MAGEA1 peptide
VLEYVIKVSA

SEQ ID NO: 161 - protein, 10 aa, Homo sapiens
  REGION 1..10: note = MAGEA1 peptide
LEYVIKVSAR

SEQ ID NO: 162 - protein, 10 aa, Homo sapiens
  REGION 1..10: note = MAGEA1 peptide
ARVRFFFPSL

SEQ ID NO: 163 - protein, 10 aa, Homo sapiens
  REGION 1..10: note = MAGEA1 peptide
RVRFFFPSLR

SEQ ID NO: 164 - protein, 10 aa, Homo sapiens
  REGION 1..10: note = MAGEA1 peptide
VKVLEYVIKV

SEQ ID NO: 165 - protein, 10 aa, Homo sapiens
  REGION 1..10: note = MAGEA1 peptide
KVLEYVIKVS

SEQ ID NO: 166 - protein, 10 aa, Homo sapiens
  REGION 1..10: note = MAGEA1 peptide
SLFRAVITKK

SEQ ID NO: 167 - protein, 10 aa, Homo sapiens
  REGION 1..10: note = MAGEA1 peptide
ESLFRAVITK

SEQ ID NO: 168 - protein, 9 aa, Homo sapiens
  REGION 1..9: note = MAGEA1 peptide
LFRAVITKK

SEQ ID NO: 169-170 - skipped (2 entries)

SEQ ID NO: 171 - protein, 7 aa, Homo sapiens
  REGION 1..7: note = TCR56 TRA CDR1
TSESDYY

SEQ ID NO: 172 - protein, 8 aa, Homo sapiens
  REGION 1..8: note = TCR56 TRA CDR2
QEAYKQQN

SEQ ID NO: 173 - protein, 14 aa, Homo sapiens
  REGION 1..14: note = TCR56 TRA CDR3
AYCRGSNFGNEKLT

SEQ ID NO: 174 - protein, 138 aa, Homo sapiens
  REGION 1..138: note = TCR56 TRA variable region (TRAV-CDR3-TRAJ) (aa)
MACPGFLWALVISTCLEFSMAQTVTQSQPEMSVQEAETVTLSCTYDTSESDYYLFWYKQPPSRQMILVIRQEAYKQQNATENRFSVNFQKAAKSFSLKISDSQLGDAAMYFCAYCRGSNFGNEKLTFGTGTRLTIIPN

SEQ ID NO: 175 - DNA, 414 bp, Homo sapiens
  misc_feature 1..414: note = TCR56 TRA variable region (TRAV-CDR3-TRAJ) (na)
  source 1..414: mol_type = other DNA
atggcctgtcctggatttctgtgggccctcgtgatcagcacctgtctcgagtttagcatggcccagaccgtgacacagtcccagcctgagatgtctgtgcaagaggccgagactgtgaccctgagctgcacctacgataccagcgagagcgactactacctgttctggtacaagcagcctcctagccggcagatgatcctggtcatcagacaagaggcctataagcagcagaacgccaccgagaacagattcagcgtgaacttccagaaggccgccaagagcttcagcctgaagatcagcgatagccagctgggcgacgccgccatgtacttttgtgcctactgccggggcagcaacttcggcaatgagaagctgaccttcggcaccggcaccaggctgacaatcatccccaac

SEQ ID NO: 176 - protein, 5 aa, Homo sapiens
  REGION 1..5: note = TCR56 TRB CDR1
MNHEY

SEQ ID NO: 177 - protein, 6 aa, Homo sapiens
  REGION 1..6: note = TCR56 TRB CDR2
SMNVEV

SEQ ID NO: 178 - protein, 13 aa, Homo sapiens
  REGION 1..13: note = TCR56 TRB CDR3
ASSLGTTNTGELF

SEQ ID NO: 179 - protein, 133 aa, Homo sapiens
  REGION 1..133: note = TCR56 TRB variable region (TRBV-CDR3-TRBJ) (aa)
MGPQLLGYVVLCLLGAGPLEAQVTQNPRYLITVTGKKLTVTCSQNMNHEYMSWYRQDPGLGLRQIYYSMNVEVTDKGDVPEGYKVSRKEKRNFPLILESPSPNQTSLYFCASSLGTTNTGELFFGEGSRLTVL

SEQ ID NO: 180 - DNA, 400 bp, Homo sapiens
  misc_feature 1..400: note = TCR56 TRB variable region (TRBV-CDR3-TRBJ) (na)
  source 1..400: mol_type = other DNA
atgggacctcaactgctgggatatgtggtgctgtgtctgctcggagccggacctctggaagctcaagtgacacagaaccccagatacctgatcaccgtgaccggcaagaaactgaccgtgacctgcagccagaacatgaaccacgagtacatgagctggtacagacaggaccctggcctgggcctgagacagatctactacagcatgaacgtggaagtgaccgacaagggcgacgtgcccgagggctacaaggtgtccagaaaagagaagcggaacttcccactgatcctggaaagcccatctcctaaccagaccagcctgtacttctgcgcctctagcctgggcaccacaaataccggcgagctgttctttggcgagggcagcagactgacagtgctgg

SEQ ID NO: 181 - protein, 5 aa, Homo sapiens
  REGION 1..5: note = TCR59 TRA CDR1
TSINN

SEQ ID NO: 182 - protein, 7 aa, Homo sapiens
  REGION 1..7: note = TCR59 TRA CDR2
IRSNERE

SEQ ID NO: 183 - protein, 12 aa, Homo sapiens
  REGION 1..12: note = TCR59 TRA CDR3
ATDPTGTASKLT

SEQ ID NO: 184 - protein, 133 aa, Homo sapiens
  REGION 1..133: note = TCR59 TRA variable region (TRAV-CDR3-TRAJ) (aa)
METLLGVSLVILWLQLARVNSQQGEEDPQALSIQEGENATMNCSYKTSINNLQWYRQNSGRGLVHLILIRSNEREKHSGRLRVTLDTSKKSSSLLITASRAADTASYFCATDPTGTASKLTFGTGTRLQVTLD

SEQ ID NO: 185 - DNA, 399 bp, Homo sapiens
  misc_feature 1..399: note = TCR59 TRA variable region (TRAV-CDR3-TRAJ) (na)
  source 1..399: mol_type = other DNA
atggaaacactgctgggcgtgtccctggtcatcctgtggctgcaactggctagagtgaacagccagcaaggcgaggaagatcctcaggctctgagcatccaagagggcgagaacgccaccatgaactgcagctacaagaccagcatcaacaacctgcagtggtacaggcagaacagcggcagaggactggtgcacctgatcctgatcagaagcaacgagagagagaagcactccggacggctgagagtgaccctggacacaagcaagaagtccagctctctgctgatcaccgccagcagagccgccgatacagccagctacttctgtgccacagatcctaccggcaccgcctccaagctgacatttggcacaggcaccaggctgcaagtgacactggat

SEQ ID NO: 186 - protein, 5 aa, Homo sapiens
  REGION 1..5: note = TCR59 TRB CDR1
SEHNR

SEQ ID NO: 187 - protein, 6 aa, Homo sapiens
  REGION 1..6: note = TCR59 TRB CDR2
FQNEAQ

SEQ ID NO: 188 - protein, 11 aa, Homo sapiens
  REGION 1..11: note = TCR59 TRB CDR3
ASSSGPYNEQF

SEQ ID NO: 189 - protein, 132 aa, Homo sapiens
  REGION 1..132: note = TCR59 TRB variable region (TRBV-CDR3-TRBJ) (aa)
MGTSLLCWMALCLLGADHADTGVSQDPRHKITKRGQNVTFRCDPISEHNRLYWYRQTLGQGPEFLTYFQNEAQLEKSRLLSDRFSAERPKGSFSTLEIQRTEQGDSAMYLCASSSGPYNEQFFGPGTRLTVL

SEQ ID NO: 190 - DNA, 397 bp, Homo sapiens
  misc_feature 1..397: note = TCR59 TRB variable region (TRBV-CDR3-TRBJ) (na)
  source 1..397: mol_type = other DNA
atgggaacatctctgctttgttggatggccctgtgtctgctgggagccgatcatgccgatacgggagtgtcccaggatcctcggcacaagattaccaagcggggccagaacgtgaccttcagatgcgaccctatcagcgagcacaaccggctgtactggtacagacagacactcggccagggacctgagttcctgacctacttccagaacgaggcccagctggaaaagagcagactgctgagcgacagattcagcgccgaaagacccaagggcagcttcagcaccctggaaatccagagaaccgagcagggcgacagcgccatgtatctgtgtgcctctagcagcggcccctacaacgagcagttctttggccctggcaccagactgaccgtgctgg

SEQ ID NO: 191 - protein, 7 aa, Homo sapiens
  REGION 1..7: note = TCR66 TRA CDR1
TRDTTYY

SEQ ID NO: 192 - protein, 8 aa, Homo sapiens
  REGION 1..8: note = TCR66 TRA CDR2
RNSFDEQN

SEQ ID NO: 193 - protein, 11 aa, Homo sapiens
  REGION 1..11: note = TCR66 TRA CDR3
ALSEFRDDKII

SEQ ID NO: 194 - protein, 135 aa, Homo sapiens
  REGION 1..135: note = TCR66 TRA variable region (TRAV-CDR3-TRAJ) (aa)
MLTASLLRAVIASICVVSSMAQKVTQAQTEISVVEKEDVTLDCVYETRDTTYYLFWYKQPPSGELVFLIRRNSFDEQNEISGRYSWNFQKSTSSFNFTITASQVVDSAVYFCALSEFRDDKIIFGKGTRLHILPN

SEQ ID NO: 195 - DNA, 405 bp, Homo sapiens
  misc_feature 1..405: note = TCR66 TRA variable region (TRAV-CDR3-TRAJ) (na)
  source 1..405: mol_type = other DNA
atgctgacagcctctctgctgagagccgtgatcgccagcatctgtgtggtgtctagcatggcccagaaagtgacacaggcccagaccgagatcagcgtggtggaaaaagaagatgtgaccctggactgcgtgtacgagacacgggacaccacctactacctgttttggtacaagcagcctcctagcggcgagctggtgttcctgatcagacggaacagcttcgacgagcagaacgagatctccggccggtacagctggaacttccagaagtccacctccagcttcaacttcaccatcaccgccagccaggtggtggatagcgccgtgtatttttgcgccctgagcgagttccgggacgacaagatcatctttggcaagggcaccagactgcacatcctgcctaac

SEQ ID NO: 196 - protein, 6 aa, Homo sapiens
  REGION 1..6: note = TCR66 TRB CDR1
GTSNPN

SEQ ID NO: 197 - protein, 5 aa, Homo sapiens
  REGION 1..5: note = TCR66 TRB CDR2
SVGIG

SEQ ID NO: 198 - protein, 11 aa, Homo sapiens
  REGION 1..11: note = TCR66 TRB CDR3
AWSVASNTEAF

SEQ ID NO: 199 - protein, 129 aa, Homo sapiens
  REGION 1..129: note = TCR66 TRB variable region (TRBV-CDR3-TRBJ) (aa)
MLCSLLALLLGTFFGVRSQTIHQWPATLVQPVGSPLSLECTVEGTSNPNLYWYRQAAGRGLQLLFYSVGIGQISSEVPQNLSASRPQDRQFILSSKKLLLSDSGFYLCAWSVASNTEAFFGQGTRLTVV

SEQ ID NO: 200 - DNA, 388 bp, Homo sapiens
  misc_feature 1..388: note = TCR66 TRB variable region (TRBV-CDR3-TRBJ) (na)
  source 1..388: mol_type = other DNA
atgctttgttctctgctggctctgctgctgggcaccttctttggcgtcagaagccagaccatccaccagtggcctgctacactggtgcagcctgttggaagccctctgagcctggaatgtaccgtggaaggcaccagcaatcccaacctgtactggtacagacaggccgctggaagaggactgcagctgctgttttacagcgtcggcatcggccagatcagcagcgaggttccacagaatctgagcgccagcagaccccaggacagacagtttatcctgagcagcaagaagctgctgctgagcgacagcggcttctacctgtgtgcttggagcgtggcctctaacaccgaggcctttttcggccaaggcacccggctgacagtggtgg

SEQ ID NO: 201 - protein, 9 aa, Homo sapiens
  REGION 1..9: note = MAGEA1 epitope presented on C*06:02
SAYGEPRKL